European Patent Specification EP 3 310 809 B1, published October 16, 2024. Title: ANTI-CGRP ANTIBODY FORMULATION. Applicant: Eli Lilly and Company. The sequence listing filed with the application follows.

SEQUENCE LISTING (7 sequences)

SEQ ID NO: 1 - protein, 107 aa, Artificial Sequence
  Synthetic Construct
DIQMTQSPSSLSASVGDRVTITCRASKDISKYLNWYQQKPGKAPKLLIYYTSGYHSGVPSRFSGSGSGTDFTLTISSLQPEDFATYYCQQGDALPPTFGGGTKVEIK

SEQ ID NO: 2 - protein, 119 aa, Artificial Sequence
  Synthetic Construct
QVQLVQSGAEVKKPGSSVKVSCKASGYTFGNYWMQWVRQAPGQGLEWMGAIYEGTGKTVYIQKFADRVTITADKSTSTAYMELSSLRSEDTAVYYCARLSDYVSGFGYWGQGTTVTVSS

SEQ ID NO: 3 - protein, 214 aa, Artificial Sequence
  Synthetic Construct
DIQMTQSPSSLSASVGDRVTITCRASKDISKYLNWYQQKPGKAPKLLIYYTSGYHSGVPSRFSGSGSGTDFTLTISSLQPEDFATYYCQQGDALPPTFGGGTKVEIKRTVAAPSVFIFPPSDEQLKSGTASVVCLLNNFYPREAKVQWKVDNALQSGNSQESVTEQDSKDSTYSLSSTLTLSKADYEKHKVYACEVTHQGLSSPVTKSFNRGEC

SEQ ID NO: 4 - protein, 445 aa, Artificial Sequence
  Synthetic Construct
QVQLVQSGAEVKKPGSSVKVSCKASGYTFGNYWMQWVRQAPGQGLEWMGAIYEGTGKTVYIQKFADRVTITADKSTSTAYMELSSLRSEDTAVYYCARLSDYVSGFGYWGQGTTVTVSSASTKGPSVFPLAPCSRSTSESTAALGCLVKDYFPEPVTVSWNSGALTSGVHTFPAVLQSSGLYSLSSVVTVPSSSLGTKTYTCNVDHKPSNTKVDKRVESKYGPPCPPCPAPEAAGGPSVFLFPPKPKDTLMISRTPEVTCVVVDVSQEDPEVQFNWYVDGVEVHNAKTKPREEQFNSTYRVVSVLTVLHQDWLNGKEYKCKVSNKGLPSSIEKTISKAKGQPREPQVYTLPPSQEEMTKNQVSLTCLVKGFYPSDIAVEWESNGQPENNYKTTPPVLDSDGSFFLYSRLTVDKSRWQEGNVFSCSVMHEALHNHYTQKSLSLSLG

SEQ ID NO: 5 - DNA, 642 bp, Artificial Sequence
  Synthetic Construct
gacatccagatgacccagtctccatcctccctgtctgcatctgtaggagacagagtcaccatcacttgccgagcaagtaaagacatttctaagtatttaaactggtatcagcagaaaccagggaaagcccctaagctcctgatctattacacatcaggatatcactcaggagtcccatcaaggttcagtggcagtggatctgggacagatttcactctcaccatcagcagtctgcaacctgaagattttgcaacttactactgtcaacaaggtgatgcgcttcctccgacgttcggcggagggaccaaggtggagatcaaacggactgtggctgcaccatctgtcttcatcttcccgccatctgatgagcagttgaaatctggaactgcctctgttgtgtgcctgctgaataacttctatcccagagaggccaaagtacagtggaaggtggataacgccctccaatcgggtaactcccaggagagtgtcacagagcaggacagcaaggacagcacctacagcctcagcagcaccctgacgctgagcaaagcagactacgagaaacacaaagtctacgcctgcgaagtcacccatcagggcctgagctcgcccgtcacaaagagcttcaacaggggagagtgc

SEQ ID NO: 6 - DNA, 1338 bp, Artificial Sequence
  Synthetic Construct
caggtgcagctggtgcagtctggggctgaggtgaagaagcctgggtcctcagtgaaggtttcctgcaaggcatctggctacacctttggtaattactggatgcagtgggtgcgacaggcccctggacaagggcttgagtggatgggagctatttatgagggaactggtaagactgtgtacattcagaagttcgccgacagagtcaccattaccgcggacaaatccacgagcacagcctacatggagctgagcagcctgagatctgaggacacggccgtgtattactgtgcgagattaagtgattacgtctcgggatttggctactggggccaaggaaccacggtcaccgtctcctcagcctccaccaagggcccatcggtcttcccgctagcgccctgctccaggagcacctccgagagcacagccgccctgggctgcctggtcaaggactacttccccgaaccggtgacggtgtcgtggaactcaggcgccctgaccagcggcgtgcacaccttcccggctgtcctacagtcctcaggactctactccctcagcagcgtggtgaccgtgccctccagcagcttgggcacgaagacctacacctgcaacgtagatcacaagcccagcaacaccaaggtggacaagagagttgagtccaaatatggtcccccatgcccaccctgcccagcacctgaggccgccgggggaccatcagtcttcctgttccccccaaaacccaaggacactctcatgatctcccggacccctgaggtcacgtgcgtggtggtggacgtgagccaggaagaccccgaggtccagttcaactggtacgtggatggcgtggaggtgcataatgccaagacaaagccgcgggaggagcagttcaacagcacgtaccgtgtggtcagcgtcctcaccgtcctgcaccaggactggctgaacggcaaggagtacaagtgcaaggtctccaacaaaggcctcccgtcctccatcgagaaaaccatctccaaagccaaagggcagccccgagagccacaggtgtacaccctgcccccatcccaggaggagatgaccaagaaccaggtcagcctgacctgcctggtcaaaggcttctaccccagcgacatcgccgtggagtgggaaagcaatgggcagccggagaacaactacaagaccacgcctcccgtgctggactccgacggctccttcttcctctacagcaggctaaccgtggacaagagcaggtggcaggaggggaatgtcttctcatgctccgtgatgcatgaggctctgcacaaccactacacacagaagagcctctccctgtctctgggttga

SEQ ID NO: 7 - protein, 37 aa, Homo sapiens
ACDTATCVTHRLAGLLSRSGGVVKNNFVPTNVGSKAF